European Patent Application EP 4 269 443 A2, published November 1, 2023. Title: Fc VARIANTS WITH ALTERED BINDING TO FcRn. Applicant: XENCOR, INC. Application EP. The sequence listing filed with the application follows.

SEQUENCE LISTING (35 sequences)

SEQ ID NO: 1 - protein, 107 aa, Homo sapiens [sequence omitted]

SEQ ID NO: 2 - protein, 330 aa, Homo sapiens
ASTKGPSVFPLAPSSKSTSGGTAALGCLVKDYFPEPVTVSWNSGALTSGVHTFPAVLQSSGLYSLSSVVTVPSSSLGTQTYICNVNHKPSNTKVDKKVEPKSCDKTHTCPPCPAPELLGGPSVFLFPPKPKDTLMISRTPEVTCVVVDVSHEDPEVKFNWYVDGVEVHNAKTKPREEQYNSTYRVVSVLTVLHQDWLNGKEYKCKVSNKALPAPIEKTISKAKGQPREPQVYTLPPSREEMTKNQVSLTCLVKGFYPSDIAVEWESNGQPENNYKTTPPVLDSDGSFFLYSKLTVDKSRWQQGNVFSCSVMHEALHNHYTQKSLSLSPGK

SEQ ID NO: 3 - protein, 326 aa, Homo sapiens
ASTKGPSVFPLAPCSRSTSESTAALGCLVKDYFPEPVTVSWNSGALTSGVHTFPAVLQSSGLYSLSSVVTVPSSNFGTQTYTCNVDHKPSNTKVDKTVERKCCVECPPCPAPPVAGPSVFLFPPKPKDTLMISRTPEVTCVVVDVSHEDPEVQFNWYVDGVEVHNAKTKPREEQFNSTFRVVSVLTVVHQDWLNGKEYKCKVSNKGLPAPIEKTISKTKGQPREPQVYTLPPSREEMTKNQVSLTCLVKGFYPSDIAVEWESNGQPENNYKTTPPMLDSDGSFFLYSKLTVDKSRWQQGNVFSCSVMHEALHNHYTQKSLSLSPGK

SEQ ID NO: 4 - protein, 377 aa, Homo sapiens
ASTKGPSVFPLAPCSRSTSGGTAALGCLVKDYFPEPVTVSWNSGALTSGVHTFPAVLQSSGLYSLSSVVTVPSSSLGTQTYTCNVNHKPSNTKVDKRVELKTPLGDTTHTCPRCPEPKSCDTPPPCPRCPEPKSCDTPPPCPRCPEPKSCDTPPPCPRCPAPELLGGPSVFLFPPKPKDTLMISRTPEVTCVVVDVSHEDPEVQFKWYVDGVEVHNAKTKPREEQYNSTFRVVSVLTVLHQDWLNGKEYKCKVSNKALPAPIEKTISKTKGQPREPQVYTLPPSREEMTKNQVSLTCLVKGFYPSDIAVEWESSGQPENNYNTTPPMLDSDGSFFLYSKLTVDKSRWQQGNIFSCSVMHEALHNRFTQKSLSLSPGK

SEQ ID NO: 5 - protein, 327 aa, Homo sapiens
ASTKGPSVFPLAPCSRSTSESTAALGCLVKDYFPEPVTVSWNSGALTSGVHTFPAVLQSSGLYSLSSVVTVPSSSLGTKTYTCNVDHKPSNTKVDKRVESKYGPPCPSCPAPEFLGGPSVFLFPPKPKDTLMISRTPEVTCVVVDVSQEDPEVQFNWYVDGVEVHNAKTKPREEQFNSTYRVVSVLTVLHQDWLNGKEYKCKVSNKGLPSSIEKTISKAKGQPREPQVYTLPPSQEEMTKNQVSLTCLVKGFYPSDIAVEWESNGQPENNYKTTPPVLDSDGSFFLYSRLTVDKSRWQEGNVFSCSVMHEALHNHYTQKSLSLSLGK

SEQ ID NO: 6 - protein, 329 aa, synthetic construct
  REGION 1..329: note = IgG1/2 constant heavy chain (CH1-hinge-CH2-CH3))
ASTKGPSVFPLAPSSKSTSGGTAALGCLVKDYFPEPVTVSWNSGALTSGVHTFPAVLQSSGLYSLSSVVTVPSSSLGTQTYICNVNHKPSNTKVDKKVEPKSCDKTHTCPPCPAPPVAGPSVFLFPPKPKDTLMISRTPEVTCVVVDVSHEDPEVQFNWYVDGVEVHNAKTKPREEQFNSTFRVVSVLTVVHQDWLNGKEYKCKVSNKGLPAPIEKTISKTKGQPREPQVYTLPPSREEMTKNQVSLTCLVKGFYPSDIAVEWESNGQPENNYKTTPPMLDSDGSFFLYSKLTVDKSRWQQGNVFSCSVMHEALHNHYTQKSLSLSPGK

SEQ ID NO: 7 - protein, 330 aa, synthetic construct
  REGION 1..330: note = IgG1 259I/308F
ASTKGPSVFPLAPSSKSTSGGTAALGCLVKDYFPEPVTVSWNSGALTSGVHTFPAVLQSSGLYSLSSVVTVPSSSLGTQTYICNVNHKPSNTKVDKKVEPKSCDKTHTCPPCPAPELLGGPSVFLFPPKPKDTLMISRTPEITCVVVDVSHEDPEVKFNWYVDGVEVHNAKTKPREEQYNSTYRVVSVLTFLHQDWLNGKEYKCKVSNKALPAPIEKTISKAKGQPREPQVYTLPPSREEMTKNQVSLTCLVKGFYPSDIAVEWESNGQPENNYKTTPPVLDSDGSFFLYSKLTVDKSRWQQGNVFSCSVMHEALHNHYTQKSLSLSPGK

SEQ ID NO: 8 - protein, 330 aa, synthetic construct
  REGION 1..330: note = IgG1 434S/428L
ASTKGPSVFPLAPSSKSTSGGTAALGCLVKDYFPEPVTVSWNSGALTSGVHTFPAVLQSSGLYSLSSVVTVPSSSLGTQTYICNVNHKPSNTKVDKKVEPKSCDKTHTCPPCPAPELLGGPSVFLFPPKPKDTLMISRTPEVTCVVVDVSHEDPEVKFNWYVDGVEVHNAKTKPREEQYNSTYRVVSVLTVLHQDWLNGKEYKCKVSNKALPAPIEKTISKAKGQPREPQVYTLPPSREEMTKNQVSLTCLVKGFYPSDIAVEWESNGQPENNYKTTPPVLDSDGSFFLYSKLTVDKSRWQQGNVFSCSVLHEALHSHYTQKSLSLSPGK

SEQ ID NO: 9 - protein, 326 aa, synthetic construct
  REGION 1..326: note = IgG2 434S
ASTKGPSVFPLAPCSRSTSESTAALGCLVKDYFPEPVTVSWNSGALTSGVHTFPAVLQSSGLYSLSSVVTVPSSNFGTQTYTCNVDHKPSNTKVDKTVERKCCVECPPCPAPPVAGPSVFLFPPKPKDTLMISRTPEVTCVVVDVSHEDPEVQFNWYVDGVEVHNAKTKPREEQFNSTFRVVSVLTVVHQDWLNGKEYKCKVSNKGLPAPIEKTISKTKGQPREPQVYTLPPSREEMTKNQVSLTCLVKGFYPSDIAVEWESNGQPENNYKTTPPMLDSDGSFFLYSKLTVDKSRWQQGNVFSCSVMHEALHSHYTQKSLSLSPGK

SEQ ID NO: 10 - protein, 326 aa, synthetic construct
  REGION 1..326: note = IgG2 434S/428L
ASTKGPSVFPLAPCSRSTSESTAALGCLVKDYFPEPVTVSWNSGALTSGVHTFPAVLQSSGLYSLSSVVTVPSSNFGTQTYTCNVDHKPSNTKVDKTVERKCCVECPPCPAPPVAGPSVFLFPPKPKDTLMISRTPEVTCVVVDVSHEDPEVQFNWYVDGVEVHNAKTKPREEQFNSTFRVVSVLTVVHQDWLNGKEYKCKVSNKGLPAPIEKTISKTKGQPREPQVYTLPPSREEMTKNQVSLTCLVKGFYPSDIAVEWESNGQPENNYKTTPPMLDSDGSFFLYSKLTVDKSRWQQGNVFSCSVLHEALHSHYTQKSLSLSPGK

SEQ ID NO: 11 - protein, 329 aa, synthetic construct
  REGION 1..329: note = IgG1/2 434S
ASTKGPSVFPLAPSSKSTSGGTAALGCLVKDYFPEPVTVSWNSGALTSGVHTFPAVLQSSGLYSLSSVVTVPSSSLGTQTYICNVNHKPSNTKVDKKVEPKSCDKTHTCPPCPAPPVAGPSVFLFPPKPKDTLMISRTPEVTCVVVDVSHEDPEVQFNWYVDGVEVHNAKTKPREEQFNSTFRVVSVLTVVHQDWLNGKEYKCKVSNKGLPAPIEKTISKTKGQPREPQVYTLPPSREEMTKNQVSLTCLVKGFYPSDIAVEWESNGQPENNYKTTPPMLDSDGSFFLYSKLTVDKSRWQQGNVFSCSVMHEALHSHYTQKSLSLSPGK

SEQ ID NO: 12 - protein, 329 aa, synthetic construct
  REGION 1..329: note = IgG1/2 434S/428L
ASTKGPSVFPLAPSSKSTSGGTAALGCLVKDYFPEPVTVSWNSGALTSGVHTFPAVLQSSGLYSLSSVVTVPSSSLGTQTYICNVNHKPSNTKVDKKVEPKSCDKTHTCPPCPAPPVAGPSVFLFPPKPKDTLMISRTPEVTCVVVDVSHEDPEVQFNWYVDGVEVHNAKTKPREEQFNSTFRVVSVLTVVHQDWLNGKEYKCKVSNKGLPAPIEKTISKTKGQPREPQVYTLPPSREEMTKNQVSLTCLVKGFYPSDIAVEWESNGQPENNYKTTPPMLDSDGSFFLYSKLTVDKSRWQQGNVFSCSVLHEALHSHYTQKSLSLSPGK

SEQ ID NO: 13 - protein, 123 aa, synthetic construct [sequence omitted]

SEQ ID NO: 14 - protein, 107 aa, synthetic construct [sequence omitted]

SEQ ID NO: 15 - protein, 121 aa, synthetic construct [sequence omitted]

SEQ ID NO: 16 - protein, 107 aa, synthetic construct [sequence omitted]

SEQ ID NO: 17 - protein, 116 aa, synthetic construct
  REGION 1..116: note = Anti-CD25
QVQLVQSGAEVKKPGASVKVSCKASGYTFTSYRMHWVRQAPGQGLEWMGWINPSTGYTEYNQKFQGRVTITADKSISTAYMELSRLRSDDTAVYYCARGGGVFDYWGQGTLVTVSS

SEQ ID NO: 18 - protein, 106 aa, synthetic construct
  REGION 1..106: note = Anti-CD25 VL
QIVLTQSPATLSLSPGERATLSCRASSSISYMHWFQQKPGQSPQLLIYTTSNLASGVPARFSGSGSGTDYTLTISSLQPEDFAVYYCHQRSTYPLTFGSGTKLEIK

SEQ ID NO: 19 - protein, 119 aa, synthetic construct
  REGION 1..119: note = Anti-EGFR VH
QVQLQQSGPGLVKPSQTLSLTCTVSGFSLSNYGVHWVRQAPGKGLEWMGIIWSGGSTDYSTSLKSRLTISKDTSKSQVVLTMTNMDPVDTATYYCARALTYYDYEFAYWGQGTLVTVSS

SEQ ID NO: 20 - protein, 107 aa, synthetic construct
  REGION 1..107: note = Anti-EGFR VL
DIQLTQSPSSLSASVGDRVTITCRASQSISSNLHWYQQKPDQSPKLLIKYASESISGVPSRFSGSGSGTDFTLTISSLQAEDVAVYYCQQNNNWPTTFGQGTKLEIK

SEQ ID NO: 21 - protein, 121 aa, synthetic construct [sequence omitted]

SEQ ID NO: 22 - protein, 111 aa, synthetic construct [sequence omitted]

SEQ ID NO: 23 - protein, 214 aa, synthetic construct
  REGION 1..214: note = Anti-TNF light chain
DIQMTQSPSSLSASVGDRVTITCRASQGIRNYLAWYQQKPGKAPKLLIYAASTLQSGVPSRFSGSGSGTDFTLTISSLQPEDVATYYCQRYNRAPYTFGQGTKVEIKRTVAAPSVFIFPPSDEQLKSGTASVVCLLNNFYPREAKVQWKVDNALQSGNSQESVTEQDSKDSTYSLSSTLTLSKADYEKHKVYACEVTHQGLSSPVTKSFNRGEC

SEQ ID NO: 24 - protein, 451 aa, synthetic construct
  REGION 1..451: note = Anti-TNF heavy chain IgG1 259I/308F
EVQLVESGGGLVQPGRSLRLSCAASGFTFDDYAMHWVRQAPGKGLEWVSAITWNSGHIDYADSVEGRFTISRDNAKNSLYLQMNSLRAEDTAVYYCAKVSYLSTASSLDYWGQGTLVTVSSASTKGPSVFPLAPSSKSTSGGTAALGCLVKDYFPEPVTVSWNSGALTSGVHTFPAVLQSSGLYSLSSVVTVPSSSLGTQTYICNVNHKPSNTKVDKKVEPKSCDKTHTCPPCPAPELLGGPSVFLFPPKPKDTLMISRTPEITCVVVDVSHEDPEVKFNWYVDGVEVHNAKTKPREEQYNSTYRVVSVLTFLHQDWLNGKEYKCKVSNKALPAPIEKTISKAKGQPREPQVYTLPPSREEMTKNQVSLTCLVKGFYPSDIAVEWESNGQPENNYKTTPPVLDSDGSFFLYSKLTVDKSRWQQGNVFSCSVMHEALHNHYTQKSLSLSPGK

SEQ ID NO: 25 - protein, 451 aa, synthetic construct
  REGION 1..451: note = Anti-TNF heavy chain IgG1 434S/428L
EVQLVESGGGLVQPGRSLRLSCAASGFTFDDYAMHWVRQAPGKGLEWVSAITWNSGHIDYADSVEGRFTISRDNAKNSLYLQMNSLRAEDTAVYYCAKVSYLSTASSLDYWGQGTLVTVSSASTKGPSVFPLAPSSKSTSGGTAALGCLVKDYFPEPVTVSWNSGALTSGVHTFPAVLQSSGLYSLSSVVTVPSSSLGTQTYICNVNHKPSNTKVDKKVEPKSCDKTHTCPPCPAPELLGGPSVFLFPPKPKDTLMISRTPEVTCVVVDVSHEDPEVKFNWYVDGVEVHNAKTKPREEQYNSTYRVVSVLTVLHQDWLNGKEYKCKVSNKALPAPIEKTISKAKGQPREPQVYTLPPSREEMTKNQVSLTCLVKGFYPSDIAVEWESNGQPENNYKTTPPVLDSDGSFFLYSKLTVDKSRWQQGNVFSCSVLHEALHSHYTQKSLSLSPGK

SEQ ID NO: 26 - protein, 447 aa, synthetic construct
  REGION 1..447: note = Anti-TNF heavy chain IgG2 434S
EVQLVESGGGLVQPGRSLRLSCAASGFTFDDYAMHWVRQAPGKGLEWVSAITWNSGHIDYADSVEGRFTISRDNAKNSLYLQMNSLRAEDTAVYYCAKVSYLSTASSLDYWGQGTLVTVSSASTKGPSVFPLAPCSRSTSESTAALGCLVKDYFPEPVTVSWNSGALTSGVHTFPAVLQSSGLYSLSSVVTVPSSNFGTQTYTCNVDHKPSNTKVDKTVERKCCVECPPCPAPPVAGPSVFLFPPKPKDTLMISRTPEVTCVVVDVSHEDPEVQFNWYVDGVEVHNAKTKPREEQFNSTFRVVSVLTVVHQDWLNGKEYKCKVSNKGLPAPIEKTISKTKGQPREPQVYTLPPSREEMTKNQVSLTCLVKGFYPSDIAVEWESNGQPENNYKTTPPMLDSDGSFFLYSKLTVDKSRWQQGNVFSCSVMHEALHSHYTQKSLSLSPGK

SEQ ID NO: 27 - protein, 447 aa, synthetic construct
  REGION 1..447: note = Anti-TNF heavy chain IgG2 434S/428L
EVQLVESGGGLVQPGRSLRLSCAASGFTFDDYAMHWVRQAPGKGLEWVSAITWNSGHIDYADSVEGRFTISRDNAKNSLYLQMNSLRAEDTAVYYCAKVSYLSTASSLDYWGQGTLVTVSSASTKGPSVFPLAPCSRSTSESTAALGCLVKDYFPEPVTVSWNSGALTSGVHTFPAVLQSSGLYSLSSVVTVPSSNFGTQTYTCNVDHKPSNTKVDKTVERKCCVECPPCPAPPVAGPSVFLFPPKPKDTLMISRTPEVTCVVVDVSHEDPEVQFNWYVDGVEVHNAKTKPREEQFNSTFRVVSVLTVVHQDWLNGKEYKCKVSNKGLPAPIEKTISKTKGQPREPQVYTLPPSREEMTKNQVSLTCLVKGFYPSDIAVEWESNGQPENNYKTTPPMLDSDGSFFLYSKLTVDKSRWQQGNVFSCSVLHEALHSHYTQKSLSLSPGK

SEQ ID NO: 28 - protein, 450 aa, synthetic construct
  REGION 1..450: note = Anti-TNF heavy chain IgG1/2 434S
EVQLVESGGGLVQPGRSLRLSCAASGFTFDDYAMHWVRQAPGKGLEWVSAITWNSGHIDYADSVEGRFTISRDNAKNSLYLQMNSLRAEDTAVYYCAKVSYLSTASSLDYWGQGTLVTVSSASTKGPSVFPLAPSSKSTSGGTAALGCLVKDYFPEPVTVSWNSGALTSGVHTFPAVLQSSGLYSLSSVVTVPSSSLGTQTYICNVNHKPSNTKVDKKVEPKSCDKTHTCPPCPAPPVAGPSVFLFPPKPKDTLMISRTPEVTCVVVDVSHEDPEVQFNWYVDGVEVHNAKTKPREEQFNSTFRVVSVLTVVHQDWLNGKEYKCKVSNKGLPAPIEKTISKTKGQPREPQVYTLPPSREEMTKNQVSLTCLVKGFYPSDIAVEWESNGQPENNYKTTPPMLDSDGSFFLYSKLTVDKSRWQQGNVFSCSVMHEALHSHYTQKSLSLSPGK

SEQ ID NO: 29 - protein, 450 aa, synthetic construct
  REGION 1..450: note = Anti-TNF heavy chain IgG1/2 434S/428L
EVQLVESGGGLVQPGRSLRLSCAASGFTFDDYAMHWVRQAPGKGLEWVSAITWNSGHIDYADSVEGRFTISRDNAKNSLYLQMNSLRAEDTAVYYCAKVSYLSTASSLDYWGQGTLVTVSSASTKGPSVFPLAPSSKSTSGGTAALGCLVKDYFPEPVTVSWNSGALTSGVHTFPAVLQSSGLYSLSSVVTVPSSSLGTQTYICNVNHKPSNTKVDKKVEPKSCDKTHTCPPCPAPPVAGPSVFLFPPKPKDTLMISRTPEVTCVVVDVSHEDPEVQFNWYVDGVEVHNAKTKPREEQFNSTFRVVSVLTVVHQDWLNGKEYKCKVSNKGLPAPIEKTISKTKGQPREPQVYTLPPSREEMTKNQVSLTCLVKGFYPSDIAVEWESNGQPENNYKTTPPMLDSDGSFFLYSKLTVDKSRWQQGNVFSCSVLHEALHSHYTQKSLSLSPGK

SEQ ID NO: 30 - protein, 489 aa, synthetic construct
  REGION 1..489: note = Anti-TNF Fc fusion with IgG1 Fc
MAPVAVWAALAVGLELWAAAHALPAQVAFTPYAPEPGSTCRLREYYDQTAQMCCSKCSPGQHAKVFCTKTSDTVCDSCEDSTYTQLWNWVPECLSCGSRCSSDQVETQACTREQNRICTCRPGWYCALSKQEGCRLCAPLRKCRPGFGVARPGTETSDVVCKPCAPGTFSNTTSSTDICRPHQICNVVAIPGNASMDAVCTSTSPTRSMAPGAVHLPQPVSTRSQHTQPTPEPSTAPSTSFLLPMGPSPPAEGSTGDEPKSCDKTHTCPPCPAPELLGGPSVFLFPPKPKDTLMISRTPEVTCVVVDVSHEDPEVKFNWYVDGVEVHNAKTKPREEQYNSTYRVVSVLTVLHQDWLNGKEYKCKVSNKALPAPIEKTISKAKGQPREPQVYTLPPSREEMTKNQVSLTCLVKGFYPSDIAVEWESNGQPENNYKTTPPVLDSDGSFFLYSKLTVDKSRWQQGNVFSCSVMHEALHNHYTQKSLSLSPGK

SEQ ID NO: 31 - protein, 488 aa, synthetic construct
  REGION 1..488: note = Anti-TNF Fc fusion with IgG2 Fc
MAPVAVWAALAVGLELWAAAHALPAQVAFTPYAPEPGSTCRLREYYDQTAQMCCSKCSPGQHAKVFCTKTSDTVCDSCEDSTYTQLWNWVPECLSCGSRCSSDQVETQACTREQNRICTCRPGWYCALSKQEGCRLCAPLRKCRPGFGVARPGTETSDVVCKPCAPGTFSNTTSSTDICRPHQICNVVAIPGNASMDAVCTSTSPTRSMAPGAVHLPQPVSTRSQHTQPTPEPSTAPSTSFLLPMGPSPPAEGSTGDEPKSCDKTHTCPPCPAPPVAGPSVFLFPPKPKDTLMISRTPEVTCVVVDVSHEDPEVQFNWYVDGVEVHNAKTKPREEQFNSTFRVVSVLTVVHQDWLNGKEYKCKVSNKGLPAPIEKTISKTKGQPREPQVYTLPPSREEMTKNQVSLTCLVKGFYPSDIAVEWESNGQPENNYKTTPPMLDSDGSFFLYSKLTVDKSRWQQGNVFSCSVMHEALHNHYTQKSLSLSPGK

SEQ ID NO: 32 - protein, 489 aa, synthetic construct
  REGION 1..489: note = Anti-TNF Fc fusion with IgG1 259I/308F Fc
MAPVAVWAALAVGLELWAAAHALPAQVAFTPYAPEPGSTCRLREYYDQTAQMCCSKCSPGQHAKVFCTKTSDTVCDSCEDSTYTQLWNWVPECLSCGSRCSSDQVETQACTREQNRICTCRPGWYCALSKQEGCRLCAPLRKCRPGFGVARPGTETSDVVCKPCAPGTFSNTTSSTDICRPHQICNVVAIPGNASMDAVCTSTSPTRSMAPGAVHLPQPVSTRSQHTQPTPEPSTAPSTSFLLPMGPSPPAEGSTGDEPKSCDKTHTCPPCPAPELLGGPSVFLFPPKPKDTLMISRTPEITCVVVDVSHEDPEVKFNWYVDGVEVHNAKTKPREEQYNSTYRVVSVLTFLHQDWLNGKEYKCKVSNKALPAPIEKTISKAKGQPREPQVYTLPPSREEMTKNQVSLTCLVKGFYPSDIAVEWESNGQPENNYKTTPPVLDSDGSFFLYSKLTVDKSRWQQGNVFSCSVMHEALHNHYTQKSLSLSPGK

SEQ ID NO: 33 - protein, 489 aa, synthetic construct
  REGION 1..489: note = Anti-TNF Fc fusion with IgG1 428L/434S Fc
MAPVAVWAALAVGLELWAAAHALPAQVAFTPYAPEPGSTCRLREYYDQTAQMCCSKCSPGQHAKVFCTKTSDTVCDSCEDSTYTQLWNWVPECLSCGSRCSSDQVETQACTREQNRICTCRPGWYCALSKQEGCRLCAPLRKCRPGFGVARPGTETSDVVCKPCAPGTFSNTTSSTDICRPHQICNVVAIPGNASMDAVCTSTSPTRSMAPGAVHLPQPVSTRSQHTQPTPEPSTAPSTSFLLPMGPSPPAEGSTGDEPKSCDKTHTCPPCPAPELLGGPSVFLFPPKPKDTLMISRTPEVTCVVVDVSHEDPEVKFNWYVDGVEVHNAKTKPREEQYNSTYRVVSVLTVLHQDWLNGKEYKCKVSNKALPAPIEKTISKAKGQPREPQVYTLPPSREEMTKNQVSLTCLVKGFYPSDIAVEWESNGQPENNYKTTPPVLDSDGSFFLYSKLTVDKSRWQQGNVFSCSVLHEALHSHYTQKSLSLSPGK

SEQ ID NO: 34 - protein, 488 aa, synthetic construct
  REGION 1..488: note = Anti-TNF Fc fusion with IgG2 434S Fc
MAPVAVWAALAVGLELWAAAHALPAQVAFTPYAPEPGSTCRLREYYDQTAQMCCSKCSPGQHAKVFCTKTSDTVCDSCEDSTYTQLWNWVPECLSCGSRCSSDQVETQACTREQNRICTCRPGWYCALSKQEGCRLCAPLRKCRPGFGVARPGTETSDVVCKPCAPGTFSNTTSSTDICRPHQICNVVAIPGNASMDAVCTSTSPTRSMAPGAVHLPQPVSTRSQHTQPTPEPSTAPSTSFLLPMGPSPPAEGSTGDEPKSCDKTHTCPPCPAPPVAGPSVFLFPPKPKDTLMISRTPEVTCVVVDVSHEDPEVQFNWYVDGVEVHNAKTKPREEQFNSTFRVVSVLTVVHQDWLNGKEYKCKVSNKGLPAPIEKTISKTKGQPREPQVYTLPPSREEMTKNQVSLTCLVKGFYPSDIAVEWESNGQPENNYKTTPPMLDSDGSFFLYSKLTVDKSRWQQGNVFSCSVMHEALHSHYTQKSLSLSPGK

SEQ ID NO: 35 - protein, 488 aa, synthetic construct
  REGION 1..488: note = Anti-TNF Fc fusion with IgG2 428L/434S Fc
MAPVAVWAALAVGLELWAAAHALPAQVAFTPYAPEPGSTCRLREYYDQTAQMCCSKCSPGQHAKVFCTKTSDTVCDSCEDSTYTQLWNWVPECLSCGSRCSSDQVETQACTREQNRICTCRPGWYCALSKQEGCRLCAPLRKCRPGFGVARPGTETSDVVCKPCAPGTFSNTTSSTDICRPHQICNVVAIPGNASMDAVCTSTSPTRSMAPGAVHLPQPVSTRSQHTQPTPEPSTAPSTSFLLPMGPSPPAEGSTGDEPKSCDKTHTCPPCPAPPVAGPSVFLFPPKPKDTLMISRTPEVTCVVVDVSHEDPEVQFNWYVDGVEVHNAKTKPREEQFNSTFRVVSVLTVVHQDWLNGKEYKCKVSNKGLPAPIEKTISKTKGQPREPQVYTLPPSREEMTKNQVSLTCLVKGFYPSDIAVEWESNGQPENNYKTTPPMLDSDGSFFLYSKLTVDKSRWQQGNVFSCSVLHEALHSHYTQKSLSLSPGK